European Patent Application EP 4 417 694 A1, published August 21, 2024. Title: Gene Construct for Expressing mRNA. Applicant: GENOMICTREE, INC. Application KR. The sequence listing filed with the application follows.

SEQUENCE LISTING (23 sequences)

SEQ ID NO: 1 - DNA, 72 bp, synthetic construct
  misc_feature 1..72: note = Leader Sequence
  source 1..72: mol_type = other DNA
attaaaggtttataccttcccaggtaacaaaccaaccaactttcgatctcttgtagatctgttctctaaacg

SEQ ID NO: 2 - DNA, 83 bp, synthetic construct
  misc_feature 1..83: note = UTR
  source 1..83: mol_type = other DNA
attaaaggtttataccttcccaggtaacaaaccaaccaactttcgatctcttgtagatctgttctctaaacgaacaaactaaa

SEQ ID NO: 3 - DNA, 76 bp, synthetic construct
  misc_feature 1..76: note = UTR
  source 1..76: mol_type = other DNA
attaaaggtttataccttcccaggtaacaaaccaaccaactttcgatctcttgtagatctgttctctaaacgaaca

SEQ ID NO: 4 - DNA, 77 bp, synthetic construct
  misc_feature 1..77: note = UTR
  source 1..77: mol_type = other DNA
attaaaggtttataccttcccaggtaacaaaccaaccaactttcgatctcttgtagatctgttctctaaacgaactt

SEQ ID NO: 5 - DNA, 196 bp, synthetic construct
  misc_feature 1..196: note = UTR
  source 1..196: mol_type = other DNA
caatctttaatcagtgtgtaacattagggaggacttgaaagagccaccacattttcaccgaggccacgcggagtacgatcgagtgtacagtgaacaatgctagggagagctgcctatatggaagagccctaatgtgtaaaattaattttagtagtgctatccccatgtgattttaatagcttcttaggagaatgac

SEQ ID NO: 6 - DNA, 44 bp, synthetic construct
  misc_feature 1..44: note = Primer
  source 1..44: mol_type = other DNA
taatacgactcactatagggattaaaggtttataccttcccagg

SEQ ID NO: 7 - DNA, 20 bp, synthetic construct
  misc_feature 1..20: note = Primer
  source 1..20: mol_type = other DNA
tcttccttgccatgttgagt

SEQ ID NO: 8 - DNA, 22 bp, synthetic construct
  misc_feature 1..22: note = Primer
  source 1..22: mol_type = other DNA
tcaaacctcttagtaccattgg

SEQ ID NO: 9 - DNA, 23 bp, synthetic construct
  misc_feature 1..23: note = Primer
  source 1..23: mol_type = other DNA
aagactcacgttaacaatattgc

SEQ ID NO: 10 - DNA, 20 bp, synthetic construct
  misc_feature 1..20: note = Promoter
  source 1..20: mol_type = other DNA
taatacgactcactataggg

SEQ ID NO: 11 - DNA, 28 bp, synthetic construct
  misc_feature 1..28: note = Primer
  source 1..28: mol_type = other DNA
tttagtttgttcgtttagagaacagatc

SEQ ID NO: 12 - DNA, 28 bp, synthetic construct
  misc_feature 1..28: note = Primer
  source 1..28: mol_type = other DNA
caatctttaatcagtgtgtaacattagg

SEQ ID NO: 13 - DNA, 30 bp, synthetic construct
  misc_feature 1..30: note = Primer
  source 1..30: mol_type = other DNA
gtcattctcctaagaagctattaaaatcac

SEQ ID NO: 14 - DNA, 40 bp, synthetic construct
  misc_feature 1..40: note = Primer
  source 1..40: mol_type = other DNA
ctctaaacgaacaaactaaaatggtgagcaagggcgagga

SEQ ID NO: 15 - DNA, 40 bp, synthetic construct
  misc_feature 1..40: note = Primer
  source 1..40: mol_type = other DNA
tacacactgattaaagattgttacttgtacagctcgtcca

SEQ ID NO: 16 - DNA, 89 bp, synthetic construct
  misc_feature 1..89: note = Primer
  source 1..89: mol_type = other DNA
tttttttttttttttttttttttttttttttttttttttttttttttttttttttttttttttttgtcattctcctaagaagctattaa

SEQ ID NO: 17 - DNA, 40 bp, synthetic construct
  misc_feature 1..40: note = Primer
  source 1..40: mol_type = other DNA
ctctaaacgaacaaactaaacaatctttaatcagtgtgta

SEQ ID NO: 18 - DNA, 1084 bp, synthetic construct
  misc_feature 1..1084: note = Synthetic Gene Construct
  source 1..1084: mol_type = other DNA
taatacgactcactatagggattaaaggtttataccttcccaggtaacaaaccaaccaactttcgatctcttgtagatctgttctctaaacgaacaaactaaaatggtgagcaagggcgaggagctgttcaccggggtggtgcccatcctggtcgagctggacggcgacgtaaacggccacaagttcagcgtgtccggcgagggcgagggcgatgccacctacggcaagctgaccctgaagttcatctgcaccaccggcaagctgcccgtgccctggcccaccctcgtgaccaccctgacctacggcgtgcagtgcttcagccgctaccccgaccacatgaagcagcacgacttcttcaagtccgccatgcccgaaggctacgtccaggagcgcaccatcttcttcaaggacgacggcaactacaagacccgcgccgaggtgaagttcgagggcgacaccctggtgaaccgcatcgagctgaagggcatcgacttcaaggaggacggcaacatcctggggcacaagctggagtacaactacaacagccacaacgtctatatcatggccgacaagcagaagaacggcatcaaggtgaacttcaagatccgccacaacatcgaggacggcagcgtgcagctcgccgaccactaccagcagaacacccccatcggcgacggccccgtgctgctgcccgacaaccactacctgagcacccagtccgccctgagcaaagaccccaacgagaagcgcgatcacatggtcctgctggagttcgtgaccgccgccgggatcactctcggcatggacgagctgtacaagtaacaatctttaatcagtgtgtaacattagggaggacttgaaagagccaccacattttcaccgaggccacgcggagtacgatcgagtgtacagtgaacaatgctagggagagctgcctatatggaagagccctaatgtgtaaaattaattttagtagtgctatccccatgtgattttaatagcttcttaggagaatgacaaaaaaaaaaaaaaaaaaaaaaaaaaaaaaaaaaaaaaaaaaaaaaaaaaaaaaaaaaaaaaaaa

SEQ ID NO: 19 - DNA, 364 bp, synthetic construct
  misc_feature 1..364: note = Synthetic Gene Construct
  source 1..364: mol_type = other DNA
taatacgactcactatagggattaaaggtttataccttcccaggtaacaaaccaaccaactttcgatctcttgtagatctgttctctaaacgaacaaactaaacaatctttaatcagtgtgtaacattagggaggacttgaaagagccaccacattttcaccgaggccacgcggagtacgatcgagtgtacagtgaacaatgctagggagagctgcctatatggaagagccctaatgtgtaaaattaattttagtagtgctatccccatgtgattttaatagcttcttaggagaatgacaaaaaaaaaaaaaaaaaaaaaaaaaaaaaaaaaaaaaaaaaaaaaaaaaaaaaaaaaaaaaaaaa

SEQ ID NO: 20 - DNA, 1624 bp, synthetic construct
  misc_feature 1..1624: note = Synthetic Gene Construct
  source 1..1624: mol_type = other DNA
taatacgactcactatagggattaaaggtttataccttcccaggtaacaaaccaaccaactttcgatctcttgtagatctgttctctaaacgaacaaactaaaatgtctgataatggaccccaaaatcagcgaaatgcaccccgcattacgtttggtggaccctcagattcaactggcagtaaccagaatggagaacgcagtggggcgcgatcaaaacaacgtcggccccaaggtttacccaataatactgcgtcttggttcaccgctctcactcaacatggcaaggaagaccttaaattccctcgaggacaaggcgttccaattaacaccaatagcagtccagatgaccaaattggctactaccgaagagctaccagacgaattcgtggtggtgacggtaaaatgaaagatctcagtccaagatggtatttctactacctaggaactgggccagaagctggacttccctatggtgctaacaaagacggcatcatatgggttgcaactgagggagccttgaatacaccaaaagatcacattggcacccgcaatcctgctaacaatgctgcaatcgtgctacaacttcctcaaggaacaacattgccaaaaggcttctacgcagaagggagcagaggcggcagtcaagcctcttctcgttcctcatcacgtagtcgcaacagttcaagaaattcaactccaggcagcagtaggggaacttctcctgctagaatggctggcaatggcggtgatgctgctcttgctttgctgctgcttgacagattgaaccagcttgagagcaaaatgtctggtaaaggccaacaacaacaaggccaaactgtcactaagaaatctgctgctgaggcttctaagaagcctcggcaaaaacgtactgccactaaagcatacaatgtaacacaagctttcggcagacgtggtccagaacaaacccaaggaaattttggggaccaggaactaatcagacaaggaactgattacaaacattggccgcaaattgcacaatttgcccccagcgcttcagcgttcttcggaatgtcgcgcattggcatggaagtcacaccttcgggaacgtggttgacctacacaggtgccatcaaattggatgacaaagatccaaatttcaaagatcaagtcattttgctgaataagcatattgacgcatacaaaacattcccaccaacagagcctaaaaaggacaaaaagaagaaggctgatgaaactcaagccttaccgcagagacagaagaaacagcaaactgtgactcttcttcctgctgcagatttggatgatttctccaaacaattgcaacaatccatgagcagtgctgactcaactcaggcctaacaatctttaatcagtgtgtaacattagggaggacttgaaagagccaccacattttcaccgaggccacgcggagtacgatcgagtgtacagtgaacaatgctagggagagctgcctatatggaagagccctaatgtgtaaaattaattttagtagtgctatccccatgtgattttaatagcttcttaggagaatgacaaaaaaaaaaaaaaaaaaaaaaaaaaaaaaaaaaaaaaaaaaaaaaaaaaaaaaaaaaaaaaaaa

SEQ ID NO: 21 - DNA, 40 bp, synthetic construct
  misc_feature 1..40: note = Primer
  source 1..40: mol_type = other DNA
gctccgctacacatggtcattttagtttgttcgtttagag

SEQ ID NO: 22 - DNA, 40 bp, synthetic construct
  misc_feature 1..40: note = Primer
  source 1..40: mol_type = other DNA
gccgaatagcttatttgtagcaatctttaatcagtgtgta

SEQ ID NO: 23 - DNA, 895 bp, synthetic construct
  misc_feature 1..895: note = Synthetic Gene Construct
  source 1..895: mol_type = other DNA
taatacgactcactatagggattaaaggtttataccttcccaggtaacaaaccaaccaactttcgatctcttgtagatctgttctctaaacgaacaaactaaaatgaccatgtgtagcggagcgaggctggccctgctggtctatgggataatcatgcacagcagcgtctacagctcacctgccgccgccggactccggttccccgggatcaggccagaggaagaggcgtacggcgaggacggaaacccgctgccagacttcgatggctcggagccgccgggcgcagggagccccgcctccgcgccgcgcgccgccgccgcctggtaccgcccggccgggagaagagatgtcgcccacgggatccttaacgaggcctaccgcaaagtgctggaccagctgtccgccgggaagcacctgcagtcgctcgtggcccggggcgtgggtgggagcctcggcggcggcgcgggggacgacgcggagccgctctccaagcgccactcggacgggatcttcacggacagctacagccgctaccggaaacaaatggctgtcaagaaatacttggcggccgtcctagggaagaggtataaacaaagggttaaaaacaaaggacgccgaatagcttatttgtagcaatctttaatcagtgtgtaacattagggaggacttgaaagagccaccacattttcaccgaggccacgcggagtacgatcgagtgtacagtgaacaatgctagggagagctgcctatatggaagagccctaatgtgtaaaattaattttagtagtgctatccccatgtgattttaatagcttcttaggagaatgacaaaaaaaaaaaaaaaaaaaaaaaaaaaaaaaaaaaaaaaaaaaaaaaaaaaaaaaaaaaaaaaaa